European Patent Specification EP 3 833 655 B1, published June 25, 2025. Title: Cleavable Linker for Peptides synthesis. Applicant: Roche Diagnostics GmbH F. Hoffmann-La Roche AG. The sequence listing filed with the application follows.

SEQUENCE LISTING (6 sequences)

SEQ ID NO: 1 - protein, 8 aa, Artificial Sequence
  peptide sequence
KATSGGLF

SEQ ID NO: 2 - protein, 15 aa, Artificial Sequence
  peptide protein
GISFSIRFAIWIRFG

SEQ ID NO: 3 - protein, 20 aa, Artificial Sequence
  peptide protein
KKKKKGISFSIRFAIWIRFG

SEQ ID NO: 4 - protein, 9 aa, Artificial Sequence
  peptide protein
IIKKSTALL

SEQ ID NO: 5 - protein, 11 aa, Artificial Sequence
  peptide protein
AFDYLAQYHGG

SEQ ID NO: 6 - protein, 57 aa, Artificial Sequence
  peptide protein
WWWWEAAAEAAAEAAAEAAAEAAAEAAAEAAAEAAAEAAAEAAAEAAAEAAAEEEEE